European Patent Specification EP 4 004 240 B1, published March 13, 2024. Title: COMPOSITIONS AND METHODS FOR DETECTION OF EPSTEIN BARR VIRUS (EBV). Applicant: F. Hoffmann-La Roche AG Roche Diagnostics GmbH Roche Molecular Systems, Inc. The sequence listing filed with the application follows.

SEQUENCE LISTING (6 sequences)

SEQ ID NO: 1 - DNA, 24 bp, Artificial Sequence
  Forward Primer
  modified_base (24)..(24): t-Butyl Benzyl-dC
catctgttgtggtatatttcctcc

SEQ ID NO: 2 - DNA, 32 bp, Artificial Sequence
  Probe
  misc_feature (0)..(1): FAM-Thr
  misc_feature (6)..(7): BHQ-2
  misc_feature (32)..(33): Phosphate
ctgggcaagaccgtgctgtttatctcaatctt

SEQ ID NO: 3 - DNA, 19 bp, Artificial Sequence
  Reverse Primer
  modified_base (19)..(19): t-Butyl Benzyl-dA
cgctaccccgctaaagtaa

SEQ ID NO: 4 - DNA, 21 bp, Artificial Sequence
  Forward Primer
  modified_base (21)..(21): t-Butyl Benzyl-dC
gcgttggaaaacattagcgac

SEQ ID NO: 5 - DNA, 30 bp, Artificial Sequence
  Probe
  misc_feature (0)..(1): FAM-Thr
  misc_feature (6)..(7): BHQ-2
  misc_feature (30)..(31): Phosphate
ttacctggtgagcaatcagacatgcgacgg

SEQ ID NO: 6 - DNA, 22 bp, Artificial Sequence
  Reverse Primer
  modified_base (22)..(22): t-Butyl Benzyl-dA
gttgctcccattcttaggtgaa